European Patent Application EP 4 663 654 A1, published December 17, 2025. Title: 多肽及其衍生物、组合物及其应用. Applicant: 杭州先为达生物科技股份有限公司. The sequence listing filed with the application follows.

SEQUENCE LISTING (25 sequences)

SEQ ID NO: 1 - protein, 37 aa, synthetic construct
  MOD_RES 37: note = trans-Hyp
ASELSTAALGRLADFLRHSSNNLKPILPPTNVGSNTX

SEQ ID NO: 2 - protein, 37 aa, synthetic construct
  MOD_RES 37: note = trans-Hyp
ASQLSTAVLGRLADFLRHSSNNLKPILPPTNVGSNTX

SEQ ID NO: 3 - protein, 37 aa, synthetic construct
ASELSTAALGRLADFLRHFTDRDRDILPPTNVGSNTP

SEQ ID NO: 4 - protein, 37 aa, synthetic construct
ASQLSTAVLGRLADFLRHFTDRDRDILPPTNVGSNTP

SEQ ID NO: 5 - protein, 37 aa, synthetic construct
  MOD_RES 37: note = trans-Hyp
ASQLSTAATQRLADFLRHSSNNLKPILPPTNVGSNTX

SEQ ID NO: 6 - protein, 37 aa, synthetic construct
ASQLSTAATQRLADFLRHFTDRDRDILPPTNVGSNTP

SEQ ID NO: 7 - protein, 37 aa, synthetic construct
  MOD_RES 37: note = trans-Hyp
ASQLSTAVTQRLADFLRHSSNNLKPILPPTNVGSNTX

SEQ ID NO: 8 - protein, 37 aa, synthetic construct
ASQLSTAVTQRLADFLRHFTDRDRDILPPTNVGSNTP

SEQ ID NO: 9 - protein, 37 aa, synthetic construct
  MOD_RES 37: note = trans-Hyp
ASQLSTAVLQRLADFLRHSSNNLKPILPPTNVGSNTX

SEQ ID NO: 10 - protein, 37 aa, synthetic construct
ASQLSTAVLQRLADFLRHFTDRDRDILPPTNVGSNTP

SEQ ID NO: 11 - protein, 37 aa, synthetic construct
  MOD_RES 37: note = trans-Hyp
ASQLSTAATQRLADFLRHSSQQLKPILPPTNVGSNTX

SEQ ID NO: 12 - protein, 37 aa, synthetic construct
  MOD_RES 37: note = trans-Hyp
ASQLSTAATQRLADFLRHSSEELKPILPPTNVGSNTX

SEQ ID NO: 13 - protein, 37 aa, synthetic construct
  MOD_RES 37: note = trans-Hyp
ASQLSTAATQRLADFLRHSSSSLKPILPPTNVGSNTX

SEQ ID NO: 14 - protein, 37 aa, synthetic construct
  MOD_RES 22: note = NMeAsn
  MOD_RES 37: note = trans-Hyp
ASQLSTAATQRLADFLRHSSNXLKPILPPTNVGSNTX

SEQ ID NO: 15 - protein, 37 aa, synthetic construct; identical to SEQ ID NO: 14
  MOD_RES 22: note = NMeAsp
  MOD_RES 37: note = trans-Hyp

SEQ ID NO: 16 - protein, 37 aa, synthetic construct
  MOD_RES 37: note = trans-Hyp
ASQLSTAATQRLADFLRHSSQNLKPILPPTNVGSNTX

SEQ ID NO: 17 - protein, 37 aa, synthetic construct
  MOD_RES 37: note = trans-Hyp
ASQLSTAATQRLADFLRHSSENLKPILPPTNVGSNTX

SEQ ID NO: 18 - protein, 37 aa, synthetic construct
  MOD_RES 37: note = trans-Hyp
ASQLSTAATQRLADFLRHSSSNLKPILPPTNVGSNTX

SEQ ID NO: 19 - protein, 37 aa, synthetic construct
  MOD_RES 37: note = trans-Hyp
ASQLSTAATQRLADFLRHSSTNLKPILPPTNVGSNTX

SEQ ID NO: 20 - protein, 37 aa, synthetic construct
  MOD_RES 37: note = trans-Hyp
ASQLSTAATQRLADFLRHSSANLKPILPPTNVGSNTX

SEQ ID NO: 21 - protein, 37 aa, synthetic construct
  MOD_RES 37: note = trans-Hyp
ASQLSTAATQRLADFLRHSSGNLKPILPPTNVGSNTX

SEQ ID NO: 22 - protein, 37 aa, synthetic construct
  MOD_RES 37: note = trans-Hyp
ASQLSTAATQRLADFLRHSSHNLKPILPPTNVGSNTX

SEQ ID NO: 23 - protein, 37 aa, synthetic construct
  MOD_RES 37: note = trans-Hyp
ASQLSTAATQRLADFLRHSSKNLKPILPPTNVGSNTX

SEQ ID NO: 24 - protein, 37 aa, synthetic construct
  MOD_RES 37: note = trans-Hyp
ASQLSTAATQRLADFLRHSSRNLKPILPPTNVGSNTX

SEQ ID NO: 25 - protein, 37 aa, synthetic construct; identical to SEQ ID NO: 14
  MOD_RES 22: note = alphaMeAsn
  MOD_RES 37: note = trans-Hyp